European Patent Specification EP 3 635 408 B1, published April 30, 2025. Title: METHODS FOR PREDICTING THE USEFULNESS OF DISEASE SPECIFIC AMINO ACID MODIFICATIONS FOR IMMUNOTHERAPY. Applicant: BioNTech RNA Pharmaceuticals GmbH. The sequence listing filed with the application follows.

SEQUENCE LISTING (23 sequences)

SEQ ID NO: 1 - protein, 15 aa, Artificial Sequence
  Linker sequence
  REPEAT (1)..(3): Portion of sequence repeated a times, wherein a is independently a number selected from 0, 1, 2, 3, 4, 5, 6, 7, 8, 9, 10, 11, 12, 13, 14, 15, 16, 17, 18, 19, or 20
  MISC_FEATURE (1)..(15): a + b + c + d + e are different from 0 and preferably are 2 or more, 3 or more, 4 or more or 5 or more
  REPEAT (4)..(6): Portion of sequence repeated b times, wherein b is independently a number selected from 0, 1, 2, 3, 4, 5, 6, 7, 8, 9, 10, 11, 12, 13, 14, 15, 16, 17, 18, 19, or 20
  REPEAT (7)..(9): Portion of sequence repeated c times, wherein c is independently a number selected from 0, 1, 2, 3, 4, 5, 6, 7, 8, 9, 10, 11, 12, 13, 14, 15, 16, 17, 18, 19, or 20
  REPEAT (10)..(12): Portion of sequence repeated d times, wherein d is independently a number selected from 0, 1, 2, 3, 4, 5, 6, 7, 8, 9, 10, 11, 12, 13, 14, 15, 16, 17, 18, 19, or 20
  REPEAT (13)..(15): Portion of sequence repeated e times, wherein e is independently a number selected from 0, 1, 2, 3, 4, 5, 6, 7, 8, 9, 10, 11, 12, 13, 14, 15, 16, 17, 18, 19, or 20
GGSGSSGGGSSGGSG

SEQ ID NO: 2 - protein, 9 aa, Artificial Sequence
  Linker sequence
GGSGGGGSG

SEQ ID NO: 3 - protein, 9 aa, Homo sapiens
KSQREFVRR

SEQ ID NO: 4 - protein, 9 aa, Homo sapiens
MRMNQGVCC

SEQ ID NO: 5 - protein, 14 aa, Homo sapiens
KFGQGLEDQLATKS

SEQ ID NO: 6 - protein, 15 aa, Homo sapiens
GQGLEDQLAQTKSLS

SEQ ID NO: 7 - protein, 15 aa, Homo sapiens
GLEDQLAQTKSLSLD

SEQ ID NO: 8 - protein, 15 aa, Homo sapiens
EDQLAQTKSLSLDDC

SEQ ID NO: 9 - protein, 15 aa, Homo sapiens
TRLSKVFSAMLAIYS

SEQ ID NO: 10 - protein, 15 aa, Homo sapiens
KVFSAMLAIYSNKPA

SEQ ID NO: 11 - protein, 15 aa, Homo sapiens
AMLAIYSNKPALWIM

SEQ ID NO: 12 - protein, 15 aa, Homo sapiens
IYSNKPALWIMAAKW

SEQ ID NO: 13 - protein, 19 aa, Homo sapiens
ADHDLGRLHSCVMASLRAQ

SEQ ID NO: 14 - protein, 9 aa, Homo sapiens
HDLGRLHSC

SEQ ID NO: 15 - protein, 9 aa, Homo sapiens
HSCVMASLR

SEQ ID NO: 16 - protein, 15 aa, Homo sapiens
ACYGADHDLGRLHSC

SEQ ID NO: 17 - protein, 15 aa, Homo sapiens
ADHDLGRLHSCVMAS

SEQ ID NO: 18 - protein, 15 aa, Homo sapiens
LGRLHSCVMASLRAQ

SEQ ID NO: 19 - protein, 15 aa, Homo sapiens
HSCVMASLRAQSPIP

SEQ ID NO: 20 - DNA, 31 bp, Artificial Sequence
  Oligonucleotide
gccaccatgatcctaaacaaagctctgmtgc

SEQ ID NO: 21 - DNA, 33 bp, Artificial Sequence
  Oligonucleotide
tatgcgatcgctcacaakggcccytggtgtctg

SEQ ID NO: 22 - protein, 27 aa, Homo sapiens
CSPGFFKFEASESLCLECPEHTLPSPE

SEQ ID NO: 23 - protein, 18 aa, Homo sapiens
MPRSESYCFPGVTLASTP